European Patent Application EP 4 212 175 A1, published July 19, 2023. Title: HUMANIZED ANTI-C1S ANTIBODIES AND METHODS OF USE THEREOF. Applicant: Bioverativ USA Inc. Application EP. The sequence listing filed with the application follows.

SEQUENCE LISTING (27 sequences)

SEQ ID NO: 1 - protein, 15 aa, Mus musculus
KASQSVDYDGDSYMN

SEQ ID NO: 2 - protein, 7 aa, Mus musculus
DASNLES

SEQ ID NO: 3 - protein, 9 aa, Mus musculus
QQSNEDPWT

SEQ ID NO: 4 - protein, 5 aa, Mus musculus
DDYIH

SEQ ID NO: 5 - protein, 17 aa, Mus musculus
RIDPADGHTKYAPKFQV

SEQ ID NO: 6 - protein, 10 aa, Mus musculus
YGYGREVFDY

SEQ ID NO: 7 - protein, 111 aa, Mus musculus
DIVLTQSPASLAVSLGQRATISCKASQSVDYDGDSYMNWYQQKTGQPPKILIYDASNLESGIPARFSGSGSGTDFTLNIHPVEEEDAAIYYCQQSNEDPWTFGGGTKLEIK

SEQ ID NO: 8 - protein, 119 aa, Mus musculus
EVQLQQSGAELVRPGASVKLSCTASGFNIKDDYIHWVKQRPEQGLEWIGRIDPADGHTKYAPKFQVKATITADTSSNTAYLQLSSLTSEDTAVYYCARYGYGREVFDYWGQGTTLTVSS

SEQ ID NO: 9 - protein, 673 aa, Homo sapiens
EPTMYGEILSPNYPQAYPSEVEKSWDIEVPEGYGIHLYFTHLDIELSENCAYDSVQIISGDTEEGRLCGQRSSNNPHSPIVEEFQVPYNKLQVIFKSDFSNEERFTGFAAYYVATDINECTDFVDVPCSHFCNNFIGGYFCSCPPEYFLHDDMKNCGVNCSGDVFTALIGEIASPNYPKPYPENSRCEYQIRLEKGFQVVVTLRREDFDVEAADSAGNCLDSLVFVAGDRQFGPYCGHGFPGPLNIETKSNALDIIFQTDLTGQKKGWKLRYHGDPMPCPKEDTPNSVWEPAKAKYVFRDVVQITCLDGFEVVEGRVGATSFYSTCQSNGKWSNSKLKCQPVDCGIPESIENGKVEDPESTLFGSVIRYTCEEPYYYMENGGGGEYHCAGNGSWVNEVLGPELPKCVPVCGVPREPFEEKQRIIGGSDADIKNFPWQVFFDNPWAGGALINEYWVLTAAHVVEGNREPTMYVGSTSVQTSRLAKSKMLTPEHVFIHPGWKLLEVPEGRTNFDNDIALVRLKDPVKMGPTVSPICLPGTSSDYNLMDGDLGLISGWGRTEKRDRAVRLKAARLPVAPLRKCKEVKVEKPTADAEAYVFTPNMICAGGEKGMDSCKGDSGGAFAVQDPNDKTKFYAAGLVSWGPQCGTYGLYTRVKNYVDWIMKTMQENSTPRED

SEQ ID NO: 10 - protein, 119 aa, synthetic construct
  REGION 1..119: note = Synthetic polypeptide
EVQLVQSGAELKKPGASVKLSCTASGFNIKDDYIHWVKQAPGQGLEWIGRIDPADGHTKYAPKFQVKATITADTSTNTAYLQLSSLTSEDTAVYYCARYGYGREVFDYWGQGTTVTVSS

SEQ ID NO: 11 - DNA, 357 bp, synthetic construct
  misc_feature 1..357: note = Synthetic nucleotide
  source 1..357: mol_type = other DNA
gaggttcagctggtgcagtctggggctgagcttaagaagccaggggcctcagtcaagttgtcctgcacagcttctggctttaacattaaagacgactatatacactgggtgaagcaggcccctggacagggcctggagtggattggaaggattgatcctgcggatggtcatactaaatatgccccgaagttccaagtcaaggccactataactgcagacacatccaccaacacagcctacctgcagctcagcagcctgacatctgaggacactgccgtctattactgtgctagatatggttacgggagggaggtctttgactactggggccaaggcaccactgtcacagtctcctca

SEQ ID NO: 12 - protein, 119 aa, synthetic construct
  REGION 1..119: note = Synthetic polypeptide
EVQLVQSGAEVKKPGASVKLSCTASGFNIKDDYIHWVKQAPGQGLEWIGRIDPADGHTKYAPKFQVKATITADTSTNTAYLELSSLRSEDTAVYYCARYGYGREVFDYWGQGTTVTVSS

SEQ ID NO: 13 - DNA, 357 bp, synthetic construct
  misc_feature 1..357: note = Synthetic nucleotide
  source 1..357: mol_type = other DNA
gaggttcagctggtgcagtctggggctgaggtgaagaagccaggggcctcagtcaagttgtcctgcacagcttctggctttaacattaaagacgactatatacactgggtgaagcaggcccctggacagggcctggagtggattggaaggattgatcctgcggatggtcatactaaatatgccccgaagttccaagtcaaggccactataactgcagacacatccaccaacacagcctacctggagctcagcagcctgagatctgaggacactgccgtctattactgtgctagatatggttacgggagggaggtctttgactactggggccaaggcaccactgtcacagtctcctca

SEQ ID NO: 14 - protein, 119 aa, synthetic construct
  REGION 1..119: note = Synthetic polypeptide
QVQLVQSGAEVKKPGASVKLSCTASGFNIKDDYIHWVKQAPGQGLEWIGRIDPADGHTKYAPKFQVKVTITADTSTSTAYLELSSLRSEDTAVYYCARYGYGREVFDYWGQGTTVTVSS

SEQ ID NO: 15 - DNA, 357 bp, synthetic construct
  misc_feature 1..357: note = Synthetic nucleotide
  source 1..357: mol_type = other DNA
caggttcagctggtgcagtctggggctgaggtgaagaagccaggggcctcagtcaagttgtcctgcacagcttctggctttaacattaaagacgactatatacactgggtgaagcaggcccctggacagggcctggagtggattggaaggattgatcctgcggatggtcatactaaatatgccccgaagttccaagtcaaagtcactataactgcagacacatccaccagcacagcctacctggagctcagcagcctgagatctgaggacactgccgtctattactgtgctagatatggttacgggagggaggtctttgactactggggccaaggcaccactgtcacagtctcctca

SEQ ID NO: 16 - protein, 119 aa, synthetic construct
  REGION 1..119: note = Synthetic polypeptide
QVQLVQSGAEVKKPGASVKVSCTASGFNIKDDYIHWVRQAPGQGLEWIGRIDPADGHTKYAPKFQVKVTITADTSTSTAYMELSSLRSEDTAVYYCARYGYGREVFDYWGQGTTVTVSS

SEQ ID NO: 17 - DNA, 357 bp, synthetic construct
  misc_feature 1..357: note = Synthetic nucleotide
  source 1..357: mol_type = other DNA
caggttcagctggtgcagtctggggctgaggtgaagaagccaggggcctcagtcaaggtctcctgcacagcttctggctttaacattaaagacgactatatacactgggtgcgccaggcccctggacagggcctggagtggattggaaggattgatcctgcggatggtcatactaaatatgccccgaagttccaagtcaaagtcactataactgcagacacatccaccagcacagcctacatggagctcagcagcctgagatctgaggacactgccgtctattactgtgctagatatggttacgggagggaggtctttgactactggggccaaggcaccactgtcacagtctcctca

SEQ ID NO: 18 - protein, 119 aa, synthetic construct
  REGION 1..119: note = Synthetic polypeptide
QVQLVQSGAEVKKPGASVKVSCAASGFNIKDDYIHWVRQAPGQGLEWIGRIDPADGHTKYAPKFQVKVTITADTSTSTAYMELSSLRSEDTAVYYCARYGYGREVFDYWGQGTTVTVSS

SEQ ID NO: 19 - DNA, 357 bp, synthetic construct
  misc_feature 1..357: note = Synthetic nucleotide
  source 1..357: mol_type = other DNA
caggttcagctggtgcagtctggggctgaggtgaagaagccaggggcctcagtcaaggtctcctgcgcagcttctggctttaacattaaagacgactatatacactgggtgcgccaggcccctggacagggcctggagtggattggaaggattgatcctgcggatggtcatactaaatatgccccgaagttccaagtcaaagtcactataactgcagacacatccaccagcacagcctacatggagctcagcagcctgagatctgaggacactgccgtctattactgtgctagatatggttacgggagggaggtctttgactactggggccaaggcaccactgtcacagtctcctca

SEQ ID NO: 20 - protein, 111 aa, synthetic construct
  REGION 1..111: note = Synthetic polypeptide
DIVLTQSPDSLAVSLGERATISCKASQSVDYDGDSYMNWYQQKTGQPPKILIYDASNLESGIPARFSGSGSGTDFTLTISSLEEEDFAIYYCQQSNEDPWTFGGGTKVEIK

SEQ ID NO: 21 - DNA, 333 bp, synthetic construct
  misc_feature 1..333: note = Synthetic nucleotide
  source 1..333: mol_type = other DNA
gacattgtgctgacccaatctccagactctttggctgtgtctctcggggagagggccaccatctcctgcaaggccagccaaagtgttgattatgatggtgatagttatatgaactggtaccaacaaaaaacaggacagccacccaaaatcctcatttatgatgcatccaatttggaatctggcatcccagccaggtttagtggcagtgggtctgggacagacttcaccctcaccatcagcagcctggaggaggaggattttgcaatctattactgtcagcaaagtaatgaagacccgtggacgttcggtggaggcaccaaggtggaaatcaaa

SEQ ID NO: 22 - protein, 111 aa, synthetic construct
  REGION 1..111: note = Synthetic polypeptide
DIVLTQSPDSLAVSLGERATISCKASQSVDYDGDSYMNWYQQKPGQPPKILIYDASNLESGIPARFSGSGSGTDFTLTISSLEPEDFAIYYCQQSNEDPWTFGGGTKVEIK

SEQ ID NO: 23 - DNA, 333 bp, synthetic construct
  misc_feature 1..333: note = Synthetic nucleotide
  source 1..333: mol_type = other DNA
gacattgtgctgacccaatctccagactctttggctgtgtctctcggggagagggccaccatctcctgcaaggccagccaaagtgttgattatgatggtgatagttatatgaactggtaccaacaaaaaccaggacagccacccaaaatcctcatttatgatgcatccaatttggaatctggcatcccagccaggtttagtggcagtgggtctgggacagacttcaccctcaccatcagcagcctggagcctgaggattttgcaatctattactgtcagcaaagtaatgaagacccgtggacgttcggtggaggcaccaaggtggaaatcaaa

SEQ ID NO: 24 - protein, 111 aa, synthetic construct
  REGION 1..111: note = Synthetic polypeptide
DIVLTQSPDSLAVSLGERATISCKASQSVDYDGDSYMNWYQQKPGQPPKLLIYDASNLESGIPARFSGSGSGTDFTLTISSLEPEDFAVYYCQQSNEDPWTFGGGTKVEIK

SEQ ID NO: 25 - DNA, 333 bp, synthetic construct
  misc_feature 1..333: note = Synthetic nucleotide
  source 1..333: mol_type = other DNA
gacattgtgctgacccaatctccagactctttggctgtgtctctcggggagagggccaccatctcctgcaaggccagccaaagtgttgattatgatggtgatagttatatgaactggtaccaacaaaaaccaggacagccacccaaactcctcatttatgatgcatccaatttggaatctggcatcccagccaggtttagtggcagtgggtctgggacagacttcaccctcaccatcagcagcctggagcctgaggattttgcagtctattactgtcagcaaagtaatgaagacccgtggacgttcggtggaggcaccaaggtggaaatcaaa

SEQ ID NO: 26 - protein, 119 aa, synthetic construct
  REGION 1..119: note = Synthetic polypeptide
  VARIANT 5: note = Xaa can be glutamine (Q) or valine (V)
  VARIANT 11: note = Xaa can be valine (V) or leucine (L)
  VARIANT 20: note = Xaa can be leucine (L) or valine (V)
  VARIANT 23: note = Xaa can be arginine (R) or threonine (T)
  VARIANT 38: note = Xaa can be lysine (K) or arginine (R)
  VARIANT 68: note = Xaa can be valine (V) or alanine (A)
  VARIANT 77: note = Xaa can be serine (S) or asparagine (N)
  VARIANT 81: note = Xaa can be leucine (L) or methionine (M)
  VARIANT 87: note = Xaa can be arginine (R) or threonine (T)
ZVQLXQSGAEXKKPGASVKXSCXASGFNIKDDYIHWVXQAPGQGLEWIGRIDPADGHTKYAPKFQVKXTITADTSTXTAYXXLSSLXSEDTAVYYCARYGYGREVFDYWGQGTTVTVSS

SEQ ID NO: 27 - protein, 111 aa, synthetic construct
  REGION 1..111: note = Synthetic polypeptide
  VARIANT 44: note = Xaa can be threonine (T) or proline (P)
  VARIANT 84: note = Xaa can be glutamic acid (E) or proline (P)
  VARIANT 89: note = Xaa can be isoleucine (I) or valine (V)
DIVLTQSPDSLAVSLGERATISCKASQSVDYDGDSYMNWYQQKXGQPPKJLIYDASNLESGIPARFSGSGSGTDFTLTISSLEXEDFAXYYCQQSNEDPWTFGGGTKVEIK